European Patent Application EP 4 516 904 A1, published March 5, 2025. Title: 一类含核苷酸类似物的双链RNAi类似物的缀合物. Applicant: 南京明德新药研发有限公司. Application CN. The sequence listing filed with the application follows.

SEQUENCE LISTING (7 sequences)

SEQ ID NO: 1 - RNA, 18 nt, synthetic construct
  source 1..18: mol_type = other RNA; note = sense strand
  modified_base 1..2: mod_base = OTHER; note = thio; note = 2'-O-methyl
  modified_base 3..4: mod_base = OTHER; note = 2'-fluoro
  modified_base 5: mod_base = OTHER; note = 2'-O-methyl
  modified_base 6..8: mod_base = OTHER; note = 2'-fluoro
  modified_base 9..18: mod_base = OTHER; note = 2'-O-methyl
atccacaatgagagtaca

SEQ ID NO: 2 - RNA, 29 nt, synthetic construct
  source 1..29: mol_type = other RNA; note = antisense strand
  modified_base 7: mod_base = OTHER; note = 2'-O-methyl; note = thio
  modified_base 8: mod_base = OTHER; note = 2'-fluoro; note = thio
  modified_base 9..11: mod_base = OTHER; note = 2'-O-methyl
  modified_base 12: mod_base = OTHER; note = n is Z
  modified_base 13..19: mod_base = OTHER; note = 2'-O-methyl
  modified_base 20: mod_base = OTHER; note = 2'-fluoro
  modified_base 21: mod_base = OTHER; note = 2'-O-methyl
  modified_base 22: mod_base = OTHER; note = 2'-fluoro
  modified_base 23..26: mod_base = OTHER; note = 2'-O-methyl
  modified_base 27..28: mod_base = OTHER; note = 2'-O-methyl; note = thio
  modified_base 29: mod_base = OTHER; note = 2'-O-methyl
ctcacatgtacnctcattgtggatgacga

SEQ ID NO: 3 - RNA, 18 nt, synthetic construct
  source 1..18: mol_type = other RNA; note = sense strand
  modified_base 1..2: mod_base = OTHER; note = thio; note = 2'-O-methyl
  modified_base 3..4: mod_base = OTHER; note = 2'-fluoro
  modified_base 5: mod_base = OTHER; note = 2'-O-methyl
  modified_base 6..8: mod_base = OTHER; note = 2'-fluoro
  modified_base 9..13: mod_base = OTHER; note = 2'-O-methyl
  modified_base 14: mod_base = OTHER; note = 2'-fluoro
  modified_base 15..18: mod_base = OTHER; note = 2'-O-methyl
atccacaatgagagtaca

SEQ ID NO: 4 - RNA, 18 nt, synthetic construct
  source 1..18: mol_type = other RNA; note = sense strand
  modified_base 1..2: mod_base = OTHER; note = 2'-O-methyl; note = thio
  modified_base 3..4: mod_base = OTHER; note = 2'-fluoro
  modified_base 5: mod_base = OTHER; note = 2'-O-methyl
  modified_base 6..8: mod_base = OTHER; note = 2'-fluoro
  modified_base 9..11: mod_base = OTHER; note = 2'-O-methyl
  modified_base 12: mod_base = OTHER; note = 2'-fluoro
  modified_base 13..18: mod_base = OTHER; note = 2'-O-methyl
atccacaatgagagtaca

SEQ ID NO: 5 - RNA, 18 nt, synthetic construct
  source 1..18: mol_type = other RNA; note = sense strand
  modified_base 1..2: mod_base = OTHER; note = thio; note = 2'-O-methyl
  modified_base 3..4: mod_base = OTHER; note = 2'-fluoro
  modified_base 5: mod_base = OTHER; note = 2'-O-methyl
  modified_base 6..8: mod_base = OTHER; note = 2'-fluoro
  modified_base 9..18: mod_base = OTHER; note = 2'-O-methyl
atccacaatgagagtaca

SEQ ID NO: 6 - RNA, 18 nt, synthetic construct
  source 1..18: mol_type = other RNA; note = sense strand
  modified_base 1..2: mod_base = OTHER; note = 2'-O-methyl; note = thio
  modified_base 3..4: mod_base = OTHER; note = 2'-fluoro
  modified_base 5: mod_base = OTHER; note = 2'-O-methyl
  modified_base 6..8: mod_base = OTHER; note = 2'-fluoro
  modified_base 9..13: mod_base = OTHER; note = 2'-O-methyl
  modified_base 14: mod_base = OTHER; note = 2'-fluoro
  modified_base 15..18: mod_base = OTHER; note = 2'-O-methyl
atccacaatgagagtaca

SEQ ID NO: 7 - RNA, 18 nt, synthetic construct
  source 1..18: mol_type = other RNA; note = sense strand
  modified_base 1..2: mod_base = OTHER; note = 2'-O-methyl; note = thio
  modified_base 3..4: mod_base = OTHER; note = 2'-fluoro
  modified_base 5: mod_base = OTHER; note = 2'-O-methyl
  modified_base 6..8: mod_base = OTHER; note = 2'-fluoro
  modified_base 9..11: mod_base = OTHER; note = 2'-O-methyl
  modified_base 12: mod_base = OTHER; note = 2'-fluoro
  modified_base 13..18: mod_base = OTHER; note = 2'-O-methyl
atccacaatgagagtaca